European Patent Application EP 4 382 534 A1, published June 12, 2024. Title: SYNTHETIC PEPTIDE FOR USE IN AN IMMUNOMOLECULAR ASSAY. Applicant: BIOMERIEUX. The sequence listing filed with the application follows.

SEQUENCE LISTING (10 sequences)

SEQ ID NO: 1 - protein, 10 aa, synthetic construct
MRGSHHHHHH

SEQ ID NO: 2 - protein, 15 aa, synthetic construct
MRGSHHHHHHSVDES

SEQ ID NO: 3 - protein, 9 aa, synthetic construct
GKKKKKKSV

SEQ ID NO: 4 - protein, 12 aa, synthetic construct
GKKKKKKSVDES

SEQ ID NO: 5 - protein, 21 aa, synthetic construct
  MOD_RES 11..12: note = X is amino-2,4-dioxa octanoic acid
MRGSHHHHHHXXGKKKKKKSV

SEQ ID NO: 6 - protein, 22 aa, synthetic construct
  MOD_RES 11..13: note = X is amino-2,4-dioxa octanoic acid
  MOD_RES 11..13: note = X is amino-2,4-dioxa octanoic acid
MRGSHHHHHHXXXGKKKKKKSV

SEQ ID NO: 7 - protein, 30 aa, synthetic construct
  MOD_RES 16..18: note = X is amino-2,4-dioxa octanoic acid
MRGSHHHHHHSVDESXXGKKKKKKSVDESL

SEQ ID NO: 8 - protein, 31 aa, synthetic construct
MRGSHHHHHHSVDESXXXGKKKKKKSVDESL

SEQ ID NO: 9 - DNA, 30 bp, Homo sapiens
  source 1..30: mol_type = genomic DNA
taatagtatcgagcggtcagagacgacttc

SEQ ID NO: 10 - DNA, 28 bp, Homo sapiens
  source 1..28: mol_type = genomic DNA
tagctaagtggcaggatgagaagtcgtc